European Patent Application EP 4 729 068 A1, published April 22, 2026. Title: LENTIVIRAL VECTOR-BASED IMMUNOTHERAPY OF PROSTATE TUMORS. Applicant: Theravectys. Application EP. The sequence listing filed with the application follows.

SEQUENCE LISTING (83 sequences)

SEQ ID NO: 1 - protein, 286 aa, synthetic construct
MRAAPLLLARAASLSLGFLFLLFFWLDRSVLAKELKFVTLVFRHGHYELGEYIRKRYRKFLNESYKHEQVYIRSTDVDRTLMSAMTNLAALFPPEGVSIWNPILLWQPIPVHTVPLSEDQLLYLPFRNCPRFQELRLHPYKDFIATLGKLSGLHGQDLFGIWSKVYDPLYCESVHNFTLPSWATEDTMTKLRELSELSLLSLYGIHKQKEKSHMKRATQIPSYKKLIMYSAHDTTVSGLQMALDVYNGLLPPYASCHLTELYFEKGEYFVEMYYRNETQHEPYPLM

SEQ ID NO: 2 - protein, 213 aa, synthetic construct
WVPVVFLTLSVTWIGAAPLILSRIVGGWECEKHSQRGRAVCGGVLVHPQWVLTAAHCIRNKSVILLGRHSLFHPEDTGQVFQVSHSFPHPLYDMSLLKNRFLRPGDDSSHDLMLLRLGPDDMDLPTQEPALGTTCYASGWGSIEPEEFLTPKKLQCVDLHVISNDVCAQVHPQKVTKFMLCAGRWTGGSEPCALPERPSLYTKVVHYRKWIKD

SEQ ID NO: 3 - protein, 505 aa, synthetic construct
MRAAPLLLARAASLSLGFLFLLFFWLDRSVLAKELKFVTLVFRHGHYELGEYIRKRYRKFLNESYKHEQVYIRSTDVDRTLMSAMTNLAALFPPEGVSIWNPILLWQPIPVHTVPLSEDQLLYLPFRNCPRFQELRLHPYKDFIATLGKLSGLHGQDLFGIWSKVYDPLYCESVHNFTLPSWATEDTMTKLRELSELSLLSLYGIHKQKEKSHMKRATQIPSYKKLIMYSAHDTTVSGLQMALDVYNGLLPPYASCHLTELYFEKGEYFVEMYYRNETQHEPYPLMLPGPDDWVPVVFLTLSVTWIGAAPLILSRIVGGWECEKHSQRGRAVCGGVLVHPQWVLTAAHCIRNKSVILLGRHSLFHPEDTGQVFQVSHSFPHPLYDMSLLKNRFLRPGDDSSHDLMLLRLGPDDMDLPTQEPALGTTCYASGWGSIEPEEFLTPKKLQCVDLHVISNDVCAQVHPQKVTKFMLCAGRWTGGSEPCALPERPSLYTKVVHYRKWIKD

SEQ ID NO: 4 - protein, 323 aa, synthetic construct
MARGPGLAPPPLRLPLLLLVLAAVTGHTAAQDNCTCPTNKMTVCSPDGPGGRCQCRALGSGMAVDCSTLTSKCLLLKARMSAPKNARTLVRPSEHALVDNDGLYDPDCDPEGRFKARQCNQTSVCWCVNSVGVRRTDKGDLSLRCDELVRTHHILIDLRHRPTAGAFNHSDLDAELRRLFRERYRLHPKFVAAVHYEQPTIQIELRQNTSQKAAGDVDIGDAAYYFERDIKGESLFQGRGGLDLRVRGEPLQVERTLIYYLDEIPPKFSMKRLTAGLIAVIVVVVVALVAGMAVLVITNRRKSGKYKKVEIKELGELRKEPSL

SEQ ID NO: 5 - protein, 275 aa, synthetic construct
MHTAAQDNCTCPTNKMTVCSPDGPGGRCQCRALGSGMAVDCSTLTSKCLLLKARMSAPKNARTLVRPSEHALVDNDGLYDPDCDPEGRFKARQCNQTSVCWCVNSVGVRRTDKGDLSLRCDELVRTHHILIDLRHRPTAGAFNHSDLDAELRRLFRERYRLHPKFVAAVHYEQPTIQIELRQNTSQKAAGDVDIGDAAYYFERDIKGESLFQGRGGLDLRVRGEPLQVERTLIYYLDEIPPKFSMKRLTTNRRKSGKYKKVEIKELGELRKEPSL

SEQ ID NO: 6 - protein, 355 aa, synthetic construct
MAQIFVKTLTGKTITLEVEPSDTIENVKAKIQDKEGIPPDQQRLIFAGKQLEDGRTLSDYNIQKESTLHLVLRLRGVAARSHTAAQDNCTCPTNKMTVCSPDGPGGRCQCRALGSGMAVDCSTLTSKCLLLKARMSAPKNARTLVRPSEHALVDNDGLYDPDCDPEGRFKARQCNQTSVCWCVNSVGVRRTDKGDLSLRCDELVRTHHILIDLRHRPTAGAFNHSDLDAELRRLFRERYRLHPKFVAAVHYEQPTIQIELRQNTSQKAAGDVDIGDAAYYFERDIKGESLFQGRGGLDLRVRGEPLQVERTLIYYLDEIPPKFSMKRLTTNRRKSGKYKKVEIKELGELRKEPSL

SEQ ID NO: 7 - protein, 273 aa, synthetic construct
MHTAAQDNCTCPTNKMTVCSPDGPGGRCQCRALGSGMAVDCSTLTSKCLLLKARMSAPKNARTLVRPSEHALVDNDGLYDPDCDPEGRFKARQCNQTSVCWCVNSVGVRRTDKGDLSLRCDELVRTHHILIDLRHRPTAGAFNHSDLDAELRRLFRERYRLHPKFVAAVHYEQPTIQIELRQNTSQKAAGDVDIGDAAYYFERDIKGESLFQGRGGLDLRVRGEPLQVERTLIYYLDEIPPKFSMKRLTTNRRKGKYKKVEIKELGELRKEPL

SEQ ID NO: 8 - protein, 249 aa, synthetic construct
MHTAAQDNCTCPTNKMTVCSPDGPGGRCQCRALGSGMAVDCSTLTSKCLLLKARMSAPKNARTLVRPSEHALVDNDGLYDPDCDPEGRFKARQCNQTSVCWCVNSVGVRRTDKGDLSLRCDELVRTHHILIDLRHRPTAGAFNHSDLDAELRRLFRERYRLHPKFVAAVHYEQPTIQIELRQNTSQKAAGDVDIGDAAYYFERDIKGESLFQGRGGLDLRVRGEPLQVERTLIYYLDEIPPKFSMKRLT

SEQ ID NO: 9 - protein, 57 aa, synthetic construct
QMFLPSPLFFFLQLLKQSSRRLEHTFVFLANFSLMLLRYIGKKRRATRFWDPRRGTP

SEQ ID NO: 10 - protein, 57 aa, synthetic construct
QMFLPSPLFFFLQLLKQSSRRLEHTFVFLRNFSLMVLRYIGKKRRATRFWDPRRGTP

SEQ ID NO: 11 - protein, 6 aa, synthetic construct
LPGPDD

SEQ ID NO: 12 - protein, 77 aa, synthetic construct
MAQIFVKTLTGKTITLEVEPSDTIENVKAKIQDKEGIPPDQQRLIFAGKQLEDGRTLSDYNIQKESTLHLVLRLRGV

SEQ ID NO: 13 - protein, 8 aa, synthetic construct
SIINFEKL

SEQ ID NO: 14 - protein, 4 aa, synthetic construct
AAAA

SEQ ID NO: 15 - protein, 150 aa, synthetic construct
MAQIFVKTLTGKTITLEVEPSDTIENVKAKIQDKEGIPPDQQRLIFAGKQLEDGRTLSDYNIQKESTLHLVLRLRGVAAAAQMFPPSLLFFFLQLLKQSSRRLEHTFVFLANFSLMLLRYIGKKRRATRFWDPRRGTPAAAASIINFEKL

SEQ ID NO: 16 - protein, 150 aa, synthetic construct
MAQIFVKTLTGKTITLEVEPSDTIENVKAKIQDKEGIPPDQQRLIFAGKQLEDGRTLSDYNIQKESTLHLVLRLRGVAAAAQMFPPSLLFFFLQLLKQSSRRLEHTFVFLRNFSLMVLRYIGKKRRATRFWDPRRGTPAAAASIINFEKL

SEQ ID NO: 17 - DNA, 858 bp, synthetic construct
  source 1..858: mol_type = other DNA
atgagggccgcccctttgttgttggctagggccgcctccctgtccctgggcttcctgttcctgctgttcttctggctggaccggtccgtgttggccaaggagctgaagttcgtgaccctggtgtttcggcatggccactacgagttgggagaatatatccgcaagaggtaccgcaagttcctgaacgagtcttacaagcacgagcaggtttacatcaggtccaccgacgtggacaggactctcatgtccgctatgaccaacctggccgcactgttcccccccgaaggcgtgtccatctggaaccccatcctcctgtggcagcccatccccgtgcacaccgtgcccctgagcgaggaccagctgctgtacctgcccttccgcaattgcccccgtttccaggagctgagactccacccctacaaggacttcattgccaccctcggcaagttgtccggcctgcacggccaggatttgttcggcatttggtccaaagtctatgaccccctctactgcgaatccgtgcacaacttcaccctcccctcctgggccaccgaagacaccatgaccaagctgagggagctgtccgagctgagtttgctgtccctgtacggcatccacaaacagaaggagaaatcccatatgaaaagggccacccagatcccctcctacaagaaactgatcatgtactccgcccacgacaccacagtctccggcctccagatggccctcgacgtctacaacggactgctgcccccctacgcctcctgtcacctcaccgaactctacttcgaaaagggcgaatacttcgtggaaatgtactacaggaacgaaacccagcacgaaccctatcccctcatg

SEQ ID NO: 18 - DNA, 639 bp, synthetic construct
  source 1..639: mol_type = other DNA
tgggtgcctgttgtcttcctgactttgtccgtgacctggatcggcgctgcccctctgatcttgtcccggattgtgggcggctgggagtgcgaaaaacactcccagaggggccgggctgtgtgtggcggtgtgctggtgcatcctcagtgggtgctgactgctgctcattgcattaggaacaagagtgtgatcttgctggggaggcactccttgttccaccccgaggatactggtcaggtgtttcaggtgtcccattccttcccccaccccctctacgacatgtccctgctgaagaacagattcttgcgccccggcgacgactcctcccacgacttgatgctgctgcggctcggccccgacgatatggacctccccacccaggagcccgccctgggaacaacctgctacgcctccggctggggctccatcgagcccgaagagttcctcacccccaagaaactgcagtgcgttgacctgcacgtgatttccaacgacgtgtgcgcccaggtgcacccccagaaggtgaccaagttcatgctgtgcgccggcaggtggacaggcggctctgaaccctgcgccctccccgaaagaccctccctgtacaccaaagtggtgcactataggaagtggatcaaggac

SEQ ID NO: 19 - DNA, 1521 bp, synthetic construct
  source 1..1521: mol_type = other DNA
atgagggccgcccctttgttgttggctagggccgcctccctgtccctgggcttcctgttcctgctgttcttctggctggaccggtccgtgttggccaaggagctgaagttcgtgaccctggtgtttcggcatggccactacgagttgggagaatatatccgcaagaggtaccgcaagttcctgaacgagtcttacaagcacgagcaggtttacatcaggtccaccgacgtggacaggactctcatgtccgctatgaccaacctggccgcactgttcccccccgaaggcgtgtccatctggaaccccatcctcctgtggcagcccatccccgtgcacaccgtgcccctgagcgaggaccagctgctgtacctgcccttccgcaattgcccccgtttccaggagctgagactccacccctacaaggacttcattgccaccctcggcaagttgtccggcctgcacggccaggatttgttcggcatttggtccaaagtctatgaccccctctactgcgaatccgtgcacaacttcaccctcccctcctgggccaccgaagacaccatgaccaagctgagggagctgtccgagctgagtttgctgtccctgtacggcatccacaaacagaaggagaaatcccatatgaaaagggccacccagatcccctcctacaagaaactgatcatgtactccgcccacgacaccacagtctccggcctccagatggccctcgacgtctacaacggactgctgcccccctacgcctcctgtcacctcaccgaactctacttcgaaaagggcgaatacttcgtggaaatgtactacaggaacgaaacccagcacgaaccctatcccctcatgctccccggccccgacgactgggtgcctgttgtcttcctgactttgtccgtgacctggatcggcgctgcccctctgatcttgtcccggattgtgggcggctgggagtgcgaaaaacactcccagaggggccgggctgtgtgtggcggtgtgctggtgcatcctcagtgggtgctgactgctgctcattgcattaggaacaagagtgtgatcttgctggggaggcactccttgttccaccccgaggatactggtcaggtgtttcaggtgtcccattccttcccccaccccctctacgacatgtccctgctgaagaacagattcttgcgccccggcgacgactcctcccacgacttgatgctgctgcggctcggccccgacgatatggacctccccacccaggagcccgccctgggaacaacctgctacgcctccggctggggctccatcgagcccgaagagttcctcacccccaagaaactgcagtgcgttgacctgcacgtgatttccaacgacgtgtgcgcccaggtgcacccccagaaggtgaccaagttcatgctgtgcgccggcaggtggacaggcggctctgaaccctgcgccctccccgaaagaccctccctgtacaccaaagtggtgcactataggaagtggatcaaggactgataa

SEQ ID NO: 20 - DNA, 972 bp, synthetic construct
  source 1..972: mol_type = other DNA
atggctaggggacctgggctggctcctcctcctctgcgactgcctctgctgctgctggtgctggctgctgtgactggacataccgctgcccaggataactgcacctgtcccacaaataagatgaccgtgtgcagcccagacggaccaggaggcagatgccagtgtagggccctgggctccggaatggcagtggattgcagcaccctgacatccaagtgtctgctgctgaaggccagaatgtccgccccaaagaacgcacgcacactggtgcggccttctgagcacgccctggtggacaatgatggcctgtacgaccctgattgcgacccagagggcagattcaaggccaggcagtgtaaccagaccagcgtgtgctggtgcgtgaatagcgtgggcgtgcggagaacagataagggcgacctgtccctgcgctgtgatgagctggtgcggacccaccacatcctgatcgacctgaggcacaggcctacagcaggagcctttaaccactctgatctggacgcagagctgaggcgcctgttccgggagagatacaggctgcacccaaagtttgtggccgccgtgcactatgagcagcccaccatccagatcgagctgaggcagaatacatctcagaaggcagcaggcgatgtggacatcggcgatgccgcctactatttcgagagagacatcaagggagagagcctgtttcagggaaggggaggcctggatctgcgcgtgcggggagagccactgcaggtggagcgcaccctgatctactatctggacgagatcccccctaagttcagcatgaagcggctgacagccggcctgatcgccgtgatcgtggtggtggtggtggccctggtggcaggcatggccgtgctggtcatcaccaaccggagaaagtccggcaaatacaaaaaggtggaaatcaaagaactgggcgaactgcgaaaggaaccaagtctgtga

SEQ ID NO: 21 - DNA, 828 bp, synthetic construct
  source 1..828: mol_type = other DNA
atgcataccgctgcccaggataactgcacctgtcccacaaataagatgaccgtgtgcagcccagacggaccaggaggcagatgccagtgtagggccctgggctccggaatggcagtggattgcagcaccctgacatccaagtgtctgctgctgaaggccagaatgtccgccccaaagaacgcacgcacactggtgcggccttctgagcacgccctggtggacaatgatggcctgtacgaccctgattgcgacccagagggcagattcaaggccaggcagtgtaaccagaccagcgtgtgctggtgcgtgaatagcgtgggcgtgcggagaacagataagggcgacctgtccctgcgctgtgatgagctggtgcggacccaccacatcctgatcgacctgaggcacaggcctacagcaggagcctttaaccactctgatctggacgcagagctgaggcgcctgttccgggagagatacaggctgcacccaaagtttgtggccgccgtgcactatgagcagcccaccatccagatcgagctgaggcagaatacatctcagaaggcagcaggcgatgtggacatcggcgatgccgcctactatttcgagagagacatcaagggagagagcctgtttcagggaaggggaggcctggatctgcgcgtgcggggagagccactgcaggtggagcgcaccctgatctactatctggacgagatcccccctaagttcagcatgaagcggctgacaaccaaccggagaaagtccggcaaatacaaaaaggtggaaatcaaagaactgggcgaactgcgaaaggaaccaagtctgtga

SEQ ID NO: 22 - DNA, 1068 bp, synthetic construct
  source 1..1068: mol_type = other DNA
atggcccagatcttcgtgaagaccctgactggtaagaccatcactctcgaagtggagccgagtgacaccattgagaatgtcaaggcaaagatccaagacaaggaaggcatccctcctgaccagcagaggttgatctttgctgggaaacagctggaagatggacgcaccctgtctgactacaacatccagaaagagtccaccctgcacctggtcctccgtctcagaggtgtggcagcccgatcccataccgctgcccaggataactgcacctgtcccacaaataagatgaccgtgtgcagcccagacggaccaggaggcagatgccagtgtagggccctgggctccggaatggcagtggattgcagcaccctgacatccaagtgtctgctgctgaaggccagaatgtccgccccaaagaacgcacgcacactggtgcggccttctgagcacgccctggtggacaatgatggcctgtacgaccctgattgcgacccagagggcagattcaaggccaggcagtgtaaccagaccagcgtgtgctggtgcgtgaatagcgtgggcgtgcggagaacagataagggcgacctgtccctgcgctgtgatgagctggtgcggacccaccacatcctgatcgacctgaggcacaggcctacagcaggagcctttaaccactctgatctggacgcagagctgaggcgcctgttccgggagagatacaggctgcacccaaagtttgtggccgccgtgcactatgagcagcccaccatccagatcgagctgaggcagaatacatctcagaaggcagcaggcgatgtggacatcggcgatgccgcctactatttcgagagagacatcaagggagagagcctgtttcagggaaggggaggcctggatctgcgcgtgcggggagagccactgcaggtggagcgcaccctgatctactatctggacgagatcccccctaagttcagcatgaagcggctgacaaccaaccggagaaagtccggcaaatacaaaaaggtggaaatcaaagaactgggcgaactgcgaaaggaaccaagtctgtga

SEQ ID NO: 23 - DNA, 822 bp, synthetic construct
  source 1..822: mol_type = other DNA
atgcataccgctgcccaggataactgcacctgtcccacaaataagatgaccgtgtgcagcccagacggaccaggaggcagatgccagtgtagggccctgggctccggaatggcagtggattgcagcaccctgacatccaagtgtctgctgctgaaggccagaatgtccgccccaaagaacgcacgcacactggtgcggccttctgagcacgccctggtggacaatgatggcctgtacgaccctgattgcgacccagagggcagattcaaggccaggcagtgtaaccagaccagcgtgtgctggtgcgtgaatagcgtgggcgtgcggagaacagataagggcgacctgtccctgcgctgtgatgagctggtgcggacccaccacatcctgatcgacctgaggcacaggcctacagcaggagcctttaaccactctgatctggacgcagagctgaggcgcctgttccgggagagatacaggctgcacccaaagtttgtggccgccgtgcactatgagcagcccaccatccagatcgagctgaggcagaatacatctcagaaggcagcaggcgatgtggacatcggcgatgccgcctactatttcgagagagacatcaagggagagagcctgtttcagggaaggggaggcctggatctgcgcgtgcggggagagccactgcaggtggagcgcaccctgatctactatctggacgagatcccccctaagttcagcatgaagcggctgacaaccaaccggagaaagggcaaatacaaaaaggtggaaatcaaagaactgggcgaactgcgaaaggaaccactgtga

SEQ ID NO: 24 - DNA, 750 bp, synthetic construct
  source 1..750: mol_type = other DNA
atgcataccgctgcccaggataactgcacctgtcccacaaataagatgaccgtgtgcagcccagacggaccaggaggcagatgccagtgtagggccctgggctccggaatggcagtggattgcagcaccctgacatccaagtgtctgctgctgaaggccagaatgtccgccccaaagaacgcacgcacactggtgcggccttctgagcacgccctggtggacaatgatggcctgtacgaccctgattgcgacccagagggcagattcaaggccaggcagtgtaaccagaccagcgtgtgctggtgcgtgaatagcgtgggcgtgcggagaacagataagggcgacctgtccctgcgctgtgatgagctggtgcggacccaccacatcctgatcgacctgaggcacaggcctacagcaggagcctttaaccactctgatctggacgcagagctgaggcgcctgttccgggagagatacaggctgcacccaaagtttgtggccgccgtgcactatgagcagcccaccatccagatcgagctgaggcagaatacatctcagaaggcagcaggcgatgtggacatcggcgatgccgcctactatttcgagagagacatcaagggagagagcctgtttcagggaaggggaggcctggatctgcgcgtgcggggagagccactgcaggtggagcgcaccctgatctactatctggacgagatcccccctaagttcagcatgaagcggctgacatga

SEQ ID NO: 25 - DNA, 171 bp, synthetic construct
  source 1..171: mol_type = other DNA
caaatgtttctgccctcccccctgttttttttcctccagttgcttaagcagtccagccgcagactggagcacacattcgtgttcctggcaaacttctcactcatgctgctgcgctacataggcaagaagaggagagccaccagattttgggacccaagacggggaacccca

SEQ ID NO: 26 - DNA, 171 bp, synthetic construct
  source 1..171: mol_type = other DNA
caaatgtttctgccctcccccctgttttttttcctccagttgcttaagcagtccagccgcagactggagcacacattcgtgttcctgaggaacttctcactcatggtgctgcgctacataggcaagaagaggagagccaccagattttgggacccaagacggggaacccca

SEQ ID NO: 27 - DNA, 18 bp, synthetic construct
  source 1..18: mol_type = other DNA
ctccccggccccgacgac

SEQ ID NO: 28 - DNA, 231 bp, synthetic construct
  source 1..231: mol_type = other DNA
atggcccagatcttcgtgaaaaccctgaccggcaagaccatcacactggaagtggaacccagcgacaccatcgagaacgtgaaggccaagatccaggacaaagagggcatccctcctgaccagcagagactgatcttcgccggaaagcagctggaagatggcagaaccctgagcgactacaacatccagaaagagtctaccctgcacctggtgctgagactgagaggcgtt

SEQ ID NO: 29 - DNA, 27 bp, synthetic construct
  source 1..27: mol_type = other DNA
agcatcatcaacttcgagaagctgtag

SEQ ID NO: 30 - DNA, 12 bp, synthetic construct
  source 1..12: mol_type = other DNA
gcagccgccgct

SEQ ID NO: 31 - DNA, 12 bp, synthetic construct
  source 1..12: mol_type = other DNA
gctgccgctgcc

SEQ ID NO: 32 - DNA, 453 bp, synthetic construct
  source 1..453: mol_type = other DNA
atggcccagatcttcgtgaaaaccctgaccggcaagaccatcacactggaagtggaacccagcgacaccatcgagaacgtgaaggccaagatccaggacaaagagggcatccctcctgaccagcagagactgatcttcgccggaaagcagctggaagatggcagaaccctgagcgactacaacatccagaaagagtctaccctgcacctggtgctgagactgagaggcgttgcagccgccgctcaaatgtttctgccctcccccctgttttttttcctccagttgcttaagcagtccagccgcagactggagcacacattcgtgttcctggcaaacttctcactcatgctgctgcgctacataggcaagaagaggagagccaccagattttgggacccaagacggggaaccccagctgccgctgccagcatcatcaacttcgagaagctgtag

SEQ ID NO: 33 - DNA, 453 bp, synthetic construct
  source 1..453: mol_type = other DNA
atggcccagatcttcgtgaaaaccctgaccggcaagaccatcacactggaagtggaacccagcgacaccatcgagaacgtgaaggccaagatccaggacaaagagggcatccctcctgaccagcagagactgatcttcgccggaaagcagctggaagatggcagaaccctgagcgactacaacatccagaaagagtctaccctgcacctggtgctgagactgagaggcgttgcagccgccgctcaaatgtttctgccctcccccctgttttttttcctccagttgcttaagcagtccagccgcagactggagcacacattcgtgttcctgaggaacttctcactcatggtgctgcgctacataggcaagaagaggagagccaccagattttgggacccaagacggggaaccccagctgccgctgccagcatcatcaacttcgagaagctgtag

SEQ ID NO: 34 - DNA, 120 bp, synthetic construct
  source 1..120: mol_type = other DNA
aattttaaaagaaaaggggggattggggggtacagtgcaggggaaagaatagtagacataatagcaacagacatacaaactaaagaattacaaaaacaaattacaaaaattcaaaatttt

SEQ ID NO: 35 - DNA, 597 bp, synthetic construct
  source 1..597: mol_type = other DNA
ttcccgataatcaacctctggattacaaaatttgtgaaagattgactggtattcttaactatgttgctccttttacgctatgtggatacgctgctttaatgcctttgtatcatgctattgcttcccgtatggctttcattttctcctccttgtataaatcctggttgctgtctctttatgaggagttgtggcccgttgtcaggcaacgtggcgtggtgtgcactgtgtttgctgacgcaacccccactggttggggcattgccaccacctgtcagctcctttccgggactttcgctttccccctccctattgccacggcggaactcatcgccgcctgccttgcccgctgctggacaggggctcggctgttgggcactgacaattccgtggtgttgtcggggaagctgacgtcctttccgcggctgctcgcctgtgttgccacctggattctgcgcgggacgtccttctgctacgtcccttcggccctcaatccagcggaccttccttcccgcggcctgctgccggctctgcggcctcttccgcgtcttcgccttcgccctcagacgagtcggatctccctttgggccgcctccccgc

SEQ ID NO: 36 - DNA, 20 bp, synthetic construct
  source 1..20: mol_type = other DNA
tggaggaggagatatgaggg

SEQ ID NO: 37 - DNA, 20 bp, synthetic construct
  source 1..20: mol_type = other DNA
ctgctgcactataccagaca

SEQ ID NO: 38 - DNA, 20 bp, synthetic construct
  source 1..20: mol_type = other DNA
tctcctctgacttcaacagc

SEQ ID NO: 39 - DNA, 20 bp, synthetic construct
  source 1..20: mol_type = other DNA
ccctgcactttttaagagcc

SEQ ID NO: 40 - DNA, 22 bp, synthetic construct
  source 1..22: mol_type = other DNA
ggatgtgaccttcctcagactc

SEQ ID NO: 41 - DNA, 22 bp, synthetic construct
  source 1..22: mol_type = other DNA
accttctcctgcgggaatccaa

SEQ ID NO: 42 - DNA, 24 bp, synthetic construct
  source 1..24: mol_type = other DNA
tcaagtggcatagatgtggaagaa

SEQ ID NO: 43 - DNA, 21 bp, synthetic construct
  source 1..21: mol_type = other DNA
tggctctgcaggattttcatg

SEQ ID NO: 44 - DNA, 25 bp, synthetic construct
  source 1..25: mol_type = other DNA
catcttctcaaaattcgagtgacaa

SEQ ID NO: 45 - DNA, 23 bp, synthetic construct
  source 1..23: mol_type = other DNA
tgggagtagacaaggtacaaccc

SEQ ID NO: 46 - DNA, 22 bp, synthetic construct
  source 1..22: mol_type = other DNA
tgacgtcactggagttgtacgg

SEQ ID NO: 47 - DNA, 21 bp, synthetic construct
  source 1..21: mol_type = other DNA
ggttcatgtcatggatggtgc

SEQ ID NO: 48 - DNA, 21 bp, synthetic construct
  source 1..21: mol_type = other DNA
tgccaccttttgacagtgatg

SEQ ID NO: 49 - DNA, 20 bp, synthetic construct
  source 1..20: mol_type = other DNA
aaggtccacgggaaagacac

SEQ ID NO: 50 - DNA, 23 bp, synthetic construct
  source 1..23: mol_type = other DNA
cctgagcaggatggagaattaca

SEQ ID NO: 51 - DNA, 19 bp, synthetic construct
  source 1..19: mol_type = other DNA
tccagaacatgccgcagag

SEQ ID NO: 52 - DNA, 21 bp, synthetic construct
  source 1..21: mol_type = other DNA
gtaccaggagccatatccacg

SEQ ID NO: 53 - DNA, 20 bp, synthetic construct
  source 1..20: mol_type = other DNA
acgagctcactctctgtggt

SEQ ID NO: 54 - DNA, 22 bp, synthetic construct
  source 1..22: mol_type = other DNA
gatgaggcttcctgtccctact

SEQ ID NO: 55 - DNA, 25 bp, synthetic construct
  source 1..25: mol_type = other DNA
tgacaggttttggaatagcatttcc

SEQ ID NO: 56 - DNA, 23 bp, synthetic construct
  source 1..23: mol_type = other DNA
ctgcaagtgcatcatcgttgttc

SEQ ID NO: 57 - DNA, 22 bp, synthetic construct
  source 1..22: mol_type = other DNA
taccacttcacaagtcggaggc

SEQ ID NO: 58 - DNA, 20 bp, synthetic construct
  source 1..20: mol_type = other DNA
cagtggagcaggtgaagagt

SEQ ID NO: 59 - DNA, 23 bp, synthetic construct
  source 1..23: mol_type = other DNA
gtccagcagactcaatacacact

SEQ ID NO: 60 - DNA, 20 bp, synthetic construct
  source 1..20: mol_type = other DNA
ggaagcacggcagcagaata

SEQ ID NO: 61 - DNA, 24 bp, synthetic construct
  source 1..24: mol_type = other DNA
aacttgagggagaagtaggaatgg

SEQ ID NO: 62 - DNA, 23 bp, synthetic construct
  source 1..23: mol_type = other DNA
gacagcctgtgttcgaggatatg

SEQ ID NO: 63 - DNA, 23 bp, synthetic construct
  source 1..23: mol_type = other DNA
tgttcttacaggagagggtagac

SEQ ID NO: 64 - DNA, 23 bp, synthetic construct
  source 1..23: mol_type = other DNA
ctactgcatgagactccgttctg

SEQ ID NO: 65 - DNA, 22 bp, synthetic construct
  source 1..22: mol_type = other DNA
agaatcccgtggataggcagag

SEQ ID NO: 66 - DNA, 20 bp, synthetic construct
  source 1..20: mol_type = other DNA
aggtccctgtcatgcttctg

SEQ ID NO: 67 - DNA, 20 bp, synthetic construct
  source 1..20: mol_type = other DNA
tctggacccattccttcttg

SEQ ID NO: 68 - DNA, 20 bp, synthetic construct
  source 1..20: mol_type = other DNA
cctctgtcacctgctcaaca

SEQ ID NO: 69 - DNA, 20 bp, synthetic construct
  source 1..20: mol_type = other DNA
gatgaattggcgtggaatct

SEQ ID NO: 70 - DNA, 19 bp, synthetic construct
  source 1..19: mol_type = other DNA
tgcaaacctaaccccgagc

SEQ ID NO: 71 - DNA, 21 bp, synthetic construct
  source 1..21: mol_type = other DNA
tctgtctgcctcttttggtca

SEQ ID NO: 72 - DNA, 20 bp, synthetic construct
  source 1..20: mol_type = other DNA
gtgcccacgtcaaggagtat

SEQ ID NO: 73 - DNA, 19 bp, synthetic construct
  source 1..19: mol_type = other DNA
gggaagctatacagggtca

SEQ ID NO: 74 - DNA, 21 bp, synthetic construct
  source 1..21: mol_type = other DNA
ctgcctcagattatctgccat

SEQ ID NO: 75 - DNA, 20 bp, synthetic construct
  source 1..20: mol_type = other DNA
aggtagcggaaggctttcac

SEQ ID NO: 76 - DNA, 18 bp, synthetic construct
  source 1..18: mol_type = other DNA
aaggcagtgatggagggg

SEQ ID NO: 77 - DNA, 19 bp, synthetic construct
  source 1..19: mol_type = other DNA
cggggtaagaacaggattg

SEQ ID NO: 78 - DNA, 20 bp, synthetic construct
  source 1..20: mol_type = other DNA
gcgttgtgtttgcttaaccg

SEQ ID NO: 79 - DNA, 20 bp, synthetic construct
  source 1..20: mol_type = other DNA
gaacactggccgttctttcc

SEQ ID NO: 80 - DNA, 20 bp, synthetic construct
  source 1..20: mol_type = other DNA
aaaatttcatcacgcccttg

SEQ ID NO: 81 - DNA, 20 bp, synthetic construct
  source 1..20: mol_type = other DNA
tctccagcttggtgaggtct

SEQ ID NO: 82 - DNA, 20 bp, synthetic construct
  source 1..20: mol_type = other DNA
tgccgtcattttctgcctca

SEQ ID NO: 83 - DNA, 20 bp, synthetic construct
  source 1..20: mol_type = other DNA
aggctcgcagggatgatttc